European Patent Application EP 4 190 145 A1, published June 7, 2023. Title: Sunflower seeds. Applicant: FUJI OIL HOLDINGS INC. The sequence listing filed with the application follows.

SEQUENCE LISTING (13 sequences)

SEQ ID NO: 1 - DNA, 586 bp, Artificial Sequence
  insert
taggggtgttcaaaaaactcgtggctcgcagctcgctcgaaactcgctcgaaaaaagctcgaagaaagctcggctcgaaattggctcggttgtaaacgagccagctcggctcggctcggtttgtaaacgagccgagctcgagcttggcctggctcggctcgtgagctcgtgagctggctcgataaggcttacatacttcatttttttttttgtcccacatcgcttagaaaacaaaaactaagggagtatctcccctataaaagaaggtaaagacaatggagaaagtgaattacctatttatacttgcatatttagccatgtggttaaattaaatggcaactatggcccttaggctttgaagaaattcatttttaagggctttttaagtaataaattttgcggtactttgttagttcgagctaaatcgagccgagccgagctagctcgaattcaaatcgagccgagctcgagcctcaaatctcagctcgatttgaaattcgagctcgagccgagccagctcgaatcgagttcgagccgagctcgagctgggtctagctcggctcgactcggctcgtttacagcccta

SEQ ID NO: 2 - DNA, 124 bp, Helianthus annuus
tatataaaacatagcaaaatataagaccatctgtgctactctcttctttctcacttgtgtggaggaaaacacaactcaaaaaactgtgcaacaacaagcacacacaagaacaacatcaacaatg

SEQ ID NO: 3 - DNA, 718 bp, Artificial Sequence
  inserted 5'UTR
tatataaaacatagcaaaatataagaccatctgtgctactcttaggggtgttcaaaaaactcgtggctcgcagctcgctcgaaactcgctcgaaaaaagctcgaagaaagctcggctcgaaattggctcggttgtaaacgagccagctcggctcggctcggtttgtaaacgagccgagctcgagcttggcctggctcggctcgtgagctcgtgagctggctcgataaggcttacatacttcatttttttttttgtcccacatcgcttagaaaacaaaaactaagggagtatctcccctataaaagaaggtaaagacaatggagaaagtgaattacctatttatacttgcatatttagccatgtggttaaattaaatggcaactatggcccttaggctttgaagaaattcatttttaagggctttttaagtaataaattttgcggtactttgttagttcgagctaaatcgagccgagccgagctagctcgaattcaaatcgagccgagctcgagcctcaaatctcagctcgatttgaaattcgagctcgagccgagccagctcgaatcgagttcgagccgagctcgagctgggtctagctcggctcgactcggctcgtttacagccctagctactctcttctttctcacttgtgtggaggaaaacacaactcaaaaaactgtgcaacaacaagcacacacaagaacaacatcaacaatg

SEQ ID NO: 4 - DNA, 29 bp, Artificial Sequence
  Primer
aacataagtctaagggcatatataaaaca

SEQ ID NO: 5 - DNA, 30 bp, Artificial Sequence
  Primer
aatttgggagatctgagaggtttcggttga

SEQ ID NO: 6 - DNA, 26 bp, Artificial Sequence
  Primer
gagtccggtgacgcttcaacgggaga

SEQ ID NO: 7 - DNA, 26 bp, Artificial Sequence
  Primer
gtggtggggtgaagggcttcttggta

SEQ ID NO: 8 - DNA, 26 bp, Artificial Sequence
  Primer
caatacggcgacgtttcaatcagacc

SEQ ID NO: 9 - DNA, 26 bp, Artificial Sequence
  Primer
ttggaggggtaaagggctttttggtg

SEQ ID NO: 10 - DNA, 20 bp, Artificial Sequence
  Primer
tcgactcggctcgtttacag

SEQ ID NO: 11 - DNA, 22 bp, Artificial Sequence
  Primer
ccattgttgatgttgttcttgt

SEQ ID NO: 12 - protein, 396 aa, Helianthus annuus
MAIRINTATFQSDLYRSFAFPQPKPLRSPKFAMASTIGSATTKVESTKKPFTPPREVHQQVLHSMPPQKIEIFKSMEGWAEDNILVHLKPVEKCWQAQDFLPDPASDGFMEQVEELRARAKEIPDDYFVVLVGDMITEEALPTYQTMLNTLDGVRDETGASPTSWAIWTRAWTAEENRHGDLLHQYLYLSGRVDMRQIQKTIQYLIGSGMDPRTENSPYLGFIYTSFQERATFISHGNTARHAKEHGDVKLAQMCGIIAADEKRHETAYTKIVEKLFEIDPDGTVLAFADMMRKKISMPAHLMYDGRDDNLFENFSAVAQRLGVYTAKDYADILEFLVGRWKVADLTGLSGEGRKAQDYVCGLAPRIRRLEERNSARAKESVNVPFSWIFDREVKL

SEQ ID NO: 13 - DNA, 1459 bp, Helianthus annuus
ctcttctttctcacttgtgtggaggaaaacacaactcaaaaaactgtgcaacaacaagcacacacaagaacaacatcaacaatggcgattcgcatcaatacggcgacgtttcaatcagacctgtatcgttcattcgcgtttcctcaaccgaaacctctcagatctcccaaattcgccatggcttccaccattggatccgctacaacgaaggttgaaagcaccaaaaagccctttacccctccaagggaggttcaccaacaggtgctacactcaatgccgccacaaaagatcgaaatcttcaaatccatggagggttgggccgaagataacatattggttcacctaaagcccgtcgaaaaatgctggcaagcacaggatttcctaccagatcccgcatctgacggatttatggaacaagtggaggaactacgagctcgggctaaggagattccggatgattactttgttgttttggtgggagatatgattactgaagaagcactgcctacttaccaaacaatgcttaatactcttgatggtgtgcgtgatgagaccggggctagccctacttcttgggctatctggactcgggcttggaccgctgaagaaaacaggcacggtgatcttctacatcagtatctgtatcttagtgggcgggtcgacatgaggcagattcagaagacaattcagtacctcattgggtctggaatggacccccggactgaaaacagtccttaccttgggttcatctacacttcatttcaagagcgtgccaccttcatctctcacggaaacacagcccggcacgcaaaggagcatggtgacgtgaagctggctcaaatgtgcggtataattgcagctgatgaaaaaaggcacgaaaccgcctacacaaaaatagtagaaaaactcttcgaaattgacccggacggcactgttctcgcttttgctgacatgatgaggaaaaagatctccatgcctgcacacttgatgtacgatgggcgtgacgataacctcttcgaaaatttctcagctgttgcccaaaggctcggtgtgtacactgcaaaggactatgcagacattctggagtttctggtgggccggtggaaggtggcggatttaaccgggctttctggtgaagggcgtaaagcccaagactatgtgtgcgggctggccccaagaatcagaaggcttgaggagaggaactcggcaagggcgaaggaaagtgtgaacgttccgttcagctggatctttgatagagaagtgaagctctgaaagttgctatagtaagttgttaaaacctatattagattgtcgtttctttcgtgtagtgctgatatgtgttttcttctcgactttgtaatgtgtctcgagttcgggtgtttgtaaacttgttggacatattataaaacttgttatgccagttttgatgacgattatcgtctcatcggtcggttgcaga